European Patent Specification EP 3 292 148 B1, published January 24, 2024. Title: Anti-Cancer fusion polypeptide. Applicant: Pieris Pharmaceuticals GmbH. Application EP 16721154.9. The sequence listing filed with the application follows.

SEQUENCE LISTING (52 sequences)

SEQ ID NO: 1 - protein, 178 aa, artificial
  negative control
QDSTSDLIPAPPLSKVPLQQNFQDNQFHGKWYVVGLAGNAILREDKDPQKMYATIYELKEDKSYNVTSVLFRKKKCDYWIRTFVPGSQPGEFTLGNIKSYPGLTSYLVRVVSTNYNQHAMVFFKKVSQNREYFKITLYGRTKELTSELKENFIRFSKSLGLPENHIVFPVPIDQCIDG

SEQ ID NO: 2 - protein, 178 aa, artificial
  positive control lipocalin mutein
QDSTSDLIPAPPLSKVPLQQNFQDNQFHGKWYVVGQAGNIRLREDKDPIKMMATIYELKEDKSYDVTMVKFDDKKCMYDIWTFVPGSQPGEFTLGKIKSFPGHTSSLVRVVSTNYNQHAMVFFKFVFQNREEFYITLYGRTKELTSELKENFIRFSKSLGLPENHIVFPVPIDQCIDG

SEQ ID NO: 3 - protein, 450 aa, artificial
  benchmark antibody heavy chain
EVQLVESGGGLVQPGGSLRLSCAASGFNIKDTYIHWVRQAPGKGLEWVARIYPTNGYTRYADSVKGRFTISADTSKNTAYLQMNSLRAEDTAVYYCSRWGGDGFYAMDYWGQGTLVTVSSASTKGPSVFPLAPSSKSTSGGTAALGCLVKDYFPEPVTVSWNSGALTSGVHTFPAVLQSSGLYSLSSVVTVPSSSLGTQTYICNVNHKPSNTKVDKKVEPKSCDKTHTCPPCPAPELLGGPSVFLFPPKPKDTLMISRTPEVTCVVVDVSHEDPEVKFNWYVDGVEVHNAKTKPREEQYNSTYRVVSVLTVLHQDWLNGKEYKCKVSNKALPAPIEKTISKAKGQPREPQVYTLPPSREEMTKNQVSLTCLVKGFYPSDIAVEWESNGQPENNYKTTPPVLDSDGSFFLYSKLTVDKSRWQQGNVFSCSVMHEALHNHYTQKSLSLSPGK

SEQ ID NO: 4 - protein, 214 aa, artificial
  benchmark antibody light chain
DIQMTQSPSSLSASVGDRVTITCRASQDVNTAVAWYQQKPGKAPKLLIYSASFLYSGVPSRFSGSRSGTDFTLTISSLQPEDFATYYCQQHYTTPPTFGQGTKVEIKRTVAAPSVFIFPPSDEQLKSGTASVVCLLNNFYPREAKVQWKVDNALQSGNSQESVTEQDSKDSTYSLSSTLTLSKADYEKHKVYACEVTHQGLSSPVTKSFNRGEC

SEQ ID NO: 5 - protein, 643 aa, artificial
  fusion polypeptide
EVQLVESGGGLVQPGGSLRLSCAASGFNIKDTYIHWVRQAPGKGLEWVARIYPTNGYTRYADSVKGRFTISADTSKNTAYLQMNSLRAEDTAVYYCSRWGGDGFYAMDYWGQGTLVTVSSASTKGPSVFPLAPSSKSTSGGTAALGCLVKDYFPEPVTVSWNSGALTSGVHTFPAVLQSSGLYSLSSVVTVPSSSLGTQTYICNVNHKPSNTKVDKKVEPKSCDKTHTCPPCPAPELLGGPSVFLFPPKPKDTLMISRTPEVTCVVVDVSHEDPEVKFNWYVDGVEVHNAKTKPREEQYNSTYRVVSVLTVLHQDWLNGKEYKCKVSNKALPAPIEKTISKAKGQPREPQVYTLPPSREEMTKNQVSLTCLVKGFYPSDIAVEWESNGQPENNYKTTPPVLDSDGSFFLYSKLTVDKSRWQQGNVFSCSVMHEALHNHYTQKSLSLSPGKGGGGSGGGGSGGGGSQDSTSDLIPAPPLSKVPLQQNFQDNQFHGKWYVVGQAGNIRLREDKDPIKMMATIYELKEDKSYDVTMVKFDDKKCMYDIWTFVPGSQPGEFTLGKIKSFPGHTSSLVRVVSTNYNQHAMVFFKFVFQNREEFYITLYGRTKELTSELKENFIRFSKSLGLPENHIVFPVPIDQCIDG

SEQ ID NO: 6 - protein, 214 aa, artificial; identical to SEQ ID NO: 4
  fusion polypeptide

SEQ ID NO: 7 - protein, 640 aa, artificial
  fusion polypeptide
EVQLVESGGGLVQPGGSLRLSCAASGFNIKDTYIHWVRQAPGKGLEWVARIYPTNGYTRYADSVKGRFTISADTSKNTAYLQMNSLRAEDTAVYYCSRWGGDGFYAMDYWGQGTLVTVSSASTKGPSVFPLAPCSRSTSESTAALGCLVKDYFPEPVTVSWNSGALTSGVHTFPAVLQSSGLYSLSSVVTVPSSSLGTKTYTCNVDHKPSNTKVDKRVESKYGPPCPPCPAPEAAGGPSVFLFPPKPKDTLMISRTPEVTCVVVDVSQEDPEVQFNWYVDGVEVHNAKTKPREEQFASTYRVVSVLTVLHQDWLNGKEYKCKVSNKGLPSSIEKTISKAKGQPREPQVYTLPPSQEEMTKNQVSLTCLVKGFYPSDIAVEWESNGQPENNYKTTPPVLDSDGSFFLYSRLTVDKSRWQEGNVFSCSVMHEALHNHYTQKSLSLSLGKGGGGSGGGGSGGGGSQDSTSDLIPAPPLSKVPLQQNFQDNQFHGKWYVVGQAGNIRLREDKDPIKMMATIYELKEDKSYDVTMVKFDDKKCMYDIWTFVPGSQPGEFTLGKIKSFPGHTSSLVRVVSTNYNQHAMVFFKFVFQNREEFYITLYGRTKELTSELKENFIRFSKSLGLPENHIVFPVPIDQCIDG

SEQ ID NO: 8 - protein, 214 aa, artificial; identical to SEQ ID NO: 4
  fusion polypeptide

SEQ ID NO: 9 - protein, 640 aa, artificial
  fusion polypeptide
EVQLVESGGGLVQPGGSLRLSCAASGFNIKDTYIHWVRQAPGKGLEWVARIYPTNGYTRYADSVKGRFTISADTSKNTAYLQMNSLRAEDTAVYYCSRWGGDGFYAMDYWGQGTLVTVSSASTKGPSVFPLAPCSRSTSESTAALGCLVKDYFPEPVTVSWNSGALTSGVHTFPAVLQSSGLYSLSSVVTVPSSSLGTKTYTCNVDHKPSNTKVDKRVESKYGPPCPPCPAPEAAGGPSVFLFPPKPKDTLMISRTPEVTCVVVDVSQEDPEVQFNWYVDGVEVHNAKTKPREEQFNSTYRVVSVLTVLHQDWLNGKEYKCKVSNKGLPSSIEKTISKAKGQPREPQVYTLPPSQEEMTKNQVSLTCLVKGFYPSDIAVEWESNGQPENNYKTTPPVLDSDGSFFLYSRLTVDKSRWQEGNVFSCSVMHEALHNHYTQKSLSLSLGKGGGGSGGGGSGGGGSQDSTSDLIPAPPLSKVPLQQNFQDNQFHGKWYVVGQAGNIRLREDKDPIKMMATIYELKEDKSYDVTMVKFDDKKCMYDIWTFVPGSQPGEFTLGKIKSFPGHTSSLVRVVSTNYNQHAMVFFKFVFQNREEFYITLYGRTKELTSELKENFIRFSKSLGLPENHIVFPVPIDQCIDG

SEQ ID NO: 10 - protein, 214 aa, artificial; identical to SEQ ID NO: 4
  fusion polypeptide

SEQ ID NO: 11 - protein, 447 aa, artificial
  fusion polypeptide
EVQLVESGGGLVQPGGSLRLSCAASGFNIKDTYIHWVRQAPGKGLEWVARIYPTNGYTRYADSVKGRFTISADTSKNTAYLQMNSLRAEDTAVYYCSRWGGDGFYAMDYWGQGTLVTVSSASTKGPSVFPLAPCSRSTSESTAALGCLVKDYFPEPVTVSWNSGALTSGVHTFPAVLQSSGLYSLSSVVTVPSSSLGTKTYTCNVDHKPSNTKVDKRVESKYGPPCPPCPAPEAAGGPSVFLFPPKPKDTLMISRTPEVTCVVVDVSQEDPEVQFNWYVDGVEVHNAKTKPREEQFNSTYRVVSVLTVLHQDWLNGKEYKCKVSNKGLPSSIEKTISKAKGQPREPQVYTLPPSQEEMTKNQVSLTCLVKGFYPSDIAVEWESNGQPENNYKTTPPVLDSDGSFFLYSRLTVDKSRWQEGNVFSCSVMHEALHNHYTQKSLSLSLGK

SEQ ID NO: 12 - protein, 407 aa, artificial
  fusion polypeptide
DIQMTQSPSSLSASVGDRVTITCRASQDVNTAVAWYQQKPGKAPKLLIYSASFLYSGVPSRFSGSRSGTDFTLTISSLQPEDFATYYCQQHYTTPPTFGQGTKVEIKRTVAAPSVFIFPPSDEQLKSGTASVVCLLNNFYPREAKVQWKVDNALQSGNSQESVTEQDSKDSTYSLSSTLTLSKADYEKHKVYACEVTHQGLSSPVTKSFNRGECGGGGSGGGGSGGGGSQDSTSDLIPAPPLSKVPLQQNFQDNQFHGKWYVVGQAGNIRLREDKDPIKMMATIYELKEDKSYDVTMVKFDDKKCMYDIWTFVPGSQPGEFTLGKIKSFPGHTSSLVRVVSTNYNQHAMVFFKFVFQNREEFYITLYGRTKELTSELKENFIRFSKSLGLPENHIVFPVPIDQCIDG

SEQ ID NO: 13 - protein, 640 aa, artificial
  fusion polypeptide
QDSTSDLIPAPPLSKVPLQQNFQDNQFHGKWYVVGQAGNIRLREDKDPIKMMATIYELKEDKSYDVTMVKFDDKKCMYDIWTFVPGSQPGEFTLGKIKSFPGHTSSLVRVVSTNYNQHAMVFFKFVFQNREEFYITLYGRTKELTSELKENFIRFSKSLGLPENHIVFPVPIDQCIDGGGGGSGGGGSGGGGSEVQLVESGGGLVQPGGSLRLSCAASGFNIKDTYIHWVRQAPGKGLEWVARIYPTNGYTRYADSVKGRFTISADTSKNTAYLQMNSLRAEDTAVYYCSRWGGDGFYAMDYWGQGTLVTVSSASTKGPSVFPLAPCSRSTSESTAALGCLVKDYFPEPVTVSWNSGALTSGVHTFPAVLQSSGLYSLSSVVTVPSSSLGTKTYTCNVDHKPSNTKVDKRVESKYGPPCPPCPAPEAAGGPSVFLFPPKPKDTLMISRTPEVTCVVVDVSQEDPEVQFNWYVDGVEVHNAKTKPREEQFNSTYRVVSVLTVLHQDWLNGKEYKCKVSNKGLPSSIEKTISKAKGQPREPQVYTLPPSQEEMTKNQVSLTCLVKGFYPSDIAVEWESNGQPENNYKTTPPVLDSDGSFFLYSRLTVDKSRWQEGNVFSCSVMHEALHNHYTQKSLSLSLGK

SEQ ID NO: 14 - protein, 214 aa, artificial; identical to SEQ ID NO: 4
  fusion polypeptide

SEQ ID NO: 15 - protein, 447 aa, artificial; identical to SEQ ID NO: 11
  fusion polypeptide

SEQ ID NO: 16 - protein, 407 aa, artificial
  fusion polypeptide
QDSTSDLIPAPPLSKVPLQQNFQDNQFHGKWYVVGQAGNIRLREDKDPIKMMATIYELKEDKSYDVTMVKFDDKKCMYDIWTFVPGSQPGEFTLGKIKSFPGHTSSLVRVVSTNYNQHAMVFFKFVFQNREEFYITLYGRTKELTSELKENFIRFSKSLGLPENHIVFPVPIDQCIDGGGGGSGGGGSGGGGSDIQMTQSPSSLSASVGDRVTITCRASQDVNTAVAWYQQKPGKAPKLLIYSASFLYSGVPSRFSGSRSGTDFTLTISSLQPEDFATYYCQQHYTTPPTFGQGTKVEIKRTVAAPSVFIFPPSDEQLKSGTASVVCLLNNFYPREAKVQWKVDNALQSGNSQESVTEQDSKDSTYSLSSTLTLSKADYEKHKVYACEVTHQGLSSPVTKSFNRGEC

SEQ ID NO: 17 - protein, 178 aa, artificial
  wildtype hNGAL
QDSTSDLIPAPPLSKVPLQQNFQDNQFQGKWYVVGLAGNAILREDKDPQKMYATIYELKEDKSYNVTSVLFRKKKCDYWIRTFVPGCQPGEFTLGNIKSYPGLTSYLVRVVSTNYNQHAMVFFKKVSQNREYFKITLYGRTKELTSELKENFIRFSKSLGLPENHIVFPVPIDQCIDG

SEQ ID NO: 18 - protein, 158 aa, artificial
  wildtype human Tlc
HHLLASDEEIQDVSGTWYLKAMTVDREFPEMNLESVTPMTLTTLEGGNLEAKVTMLISGRCQEVKAVLEKTDEPGKYTADGGKHVAYIIRSHVKDHYIFYCEGELHGKPVRGVKLVGRDPKNNLEALEDFEKAAGARGLSTESILIPRQSETCSPGSD

SEQ ID NO: 19 - protein, 15 aa, artificial
  linker
GGGGSGGGGSGGGGS

SEQ ID NO: 20 - DNA, 1929 bp, artificial
  fusion polypeptide
gaagtccagctggtcgaatctggtggtggcctggtccagcctggtggatcactgagactgtcctgtgctgcttctggtttcaacatcaaggacacctacatccattgggtcagacaggcacctggcaagggactggaatgggtcgcccgaatctaccctacaaacggctacactcgctacgccgactccgtcaagggacgctttaccatctccgccgacacctctaaaaacaccgcctacctgcagatgaatagtctgagggccgaggatactgctgtgtactactgctcacgatggggaggcgacggcttttacgctatggattactggggacagggaactctggtcactgtgtctagcgctagcacaaagggccctagtgtgtttcctctggctccctcttccaaatccacttctggtggcactgctgctctgggatgcctggtgaaggattactttcctgaacctgtgactgtctcatggaactctggtgctctgacttctggtgtccacactttccctgctgtgctgcagtctagtggactgtactctctgtcatctgtggtcactgtgccctcttcatctctgggaacccagacctacatttgtaatgtgaaccacaaaccatccaacactaaagtggacaaaaaagtggaacccaaatcctgtgacaaaacccacacctgcccaccttgtcctgcccctgaactgctgggaggaccttctgtgtttctgttcccaccaaaaccaaaagataccctgatgatctctagaacccctgaggtgacatgtgtggtggtggatgtgtctcatgaggaccctgaggtcaaattcaactggtacgtggatggagtggaagtccacaatgccaaaaccaagcctagagaggaacagtacaattcaacctacagagtggtcagtgtgctgactgtgctgcatcaggattggctgaatggcaaggaatacaagtgtaaagtctcaaacaaggccctgcctgctccaattgagaaaacaatctcaaaggccaagggacagcctagggaaccccaggtctacaccctgccaccttcaagagaggaaatgaccaaaaaccaggtgtccctgacatgcctggtcaaaggcttctacccttctgacattgctgtggagtgggagtcaaatggacagcctgagaacaactacaaaacaaccccccctgtgctggattctgatggctctttctttctgtactccaaactgactgtggacaagtctagatggcagcaggggaatgtcttttcttgctctgtcatgcatgaggctctgcataaccactacactcagaaatccctgtctctgtctcctggcaaaggcggcggaggatccgggggtgggggaagcggcggaggaggtagccaggactctactagtgatctgatcccggcaccgccactgtcaaaagtccctctgcaacaaaactttcaagacaatcagtttcacggcaaatggtatgtggtcggccaggccggaaacattaggctgcgggaggacaaggaccccatcaaaatgatggctaccatctacgagctgaaggaagacaaatcttatgatgtgacaatggtcaagttcgacgataagaaatgcatgtacgacatctggaccttcgtgcccggctcccagccgggagagttcaccctgggcaagatcaagtccttccccggccacacttccagcctggtccgcgtggtctcgaccaactataatcagcatgctatggtgttcttcaagttcgtctttcagaatagagaggagttctacatcacactgtatggacgcaccaaggagctgacaagcgagctgaaagaaaacttcatcaggttttcaaagtccctggggctgcccgaaaatcatatcgtgttcccagtccccatcgaccagtgtattgatggt

SEQ ID NO: 21 - DNA, 642 bp, artificial
  fusion polypeptide
gacatccagatgacacagtctccctcttccctgtccgcttctgtgggcgatcgagtgacaatcacctgtagggctagtcaggatgtgaatactgctgttgcttggtaccagcagaaaccaggaaaagcccctaaactgctgatctactctgcctcattcctgtactctggggtgccttctcgattcagtggttctagatctggcaccgatttcacactgaccatttcttcactgcaacctgaggattttgccacctactactgtcagcagcactacacaacacctcccacatttggccagggcacaaaagtggagatcaaacggaccgtggcggcgccttctgtgttcattttccccccatctgatgaacagctgaaatctggcactgcttctgtggtctgtctgctgaacaacttctaccctagagaggccaaagtccagtggaaagtggacaatgctctgcagagtgggaattcccaggaatctgtcactgagcaggactctaaggatagcacatactccctgtcctctactctgacactgagcaaggctgattacgagaaacacaaagtgtacgcctgtgaagtcacacatcaggggctgtctagtcctgtgaccaaatccttcaataggggagagtgc

SEQ ID NO: 22 - DNA, 1920 bp, artificial
  fusion polypeptide
gaagtccagctggtcgaatctggtggtggcctggtccagcctggtggatcactgagactgtcctgtgctgcttctggtttcaacatcaaggacacctacatccattgggtcagacaggcacctggcaagggactggaatgggtcgcccgaatctaccctacaaacggctacactcgctacgccgactccgtcaagggacgctttaccatctccgccgacacctctaaaaacaccgcctacctgcaaatgaatagtctgagggccgaggatactgctgtgtactactgctcacgatggggaggcgacggcttttacgctatggattactggggacagggaactctggtcactgtctcgagcgctagcaccaagggcccctccgtgttccccctggccccttgctcccggtccacctccgagtctaccgccgctctgggctgcctggtgaaagactacttccccgagcctgtgaccgtgagctggaactctggcgccctgacctccggcgtgcacaccttccctgccgtgctgcaatcctccggcctgtactccctgtcctccgtggtgacagtgccctcctccagcctgggcaccaagacctacacctgtaacgtggaccacaagccctccaacaccaaggtggacaagcgggtggaatctaaatacggccctccctgccccccctgccctgcccctgaagcggcgggcggaccttccgtgtttctgttccccccaaagcccaaggacaccctgatgatctcccggacccccgaagtgacctgcgtggtggtggacgtgtcccaggaagatccagaggtgcagttcaactggtatgttgacggcgtggaagtgcacaacgccaagaccaagcccagagaggaacagttcgcctccacctaccgggtggtgtccgtgctgaccgtgctgcaccaggactggctgaacggcaaagagtacaagtgcaaggtgtccaacaagggcctgccctccagcatcgaaaagaccatctccaaggccaagggccagccccgcgagccccaggtgtacaccctgccccctagccaggaagagatgaccaagaaccaggtgtccctgacctgtctggtgaaaggcttctacccctccgacattgccgtggaatgggagtccaacggccagcccgagaacaactacaagaccaccccccctgtgctggactccgacggctccttcttcctgtactctcggctgacagtggataagtcccggtggcaggaaggcaatgtgttctcctgcagcgtgatgcacgaggccctgcacaaccactatacccagaagtccctgtccctgagcctgggcaagggcggtggaggatccgggggtgggggaagcggcggaggaggtagccaggactctactagtgatctgatcccggcaccgccactgtcaaaagtccctctgcaacaaaactttcaagacaatcagtttcacggcaaatggtatgtggtcggccaggccggaaacattaggctgcgggaggacaaggaccccatcaaaatgatggctaccatctacgagctgaaggaagacaaatcttatgatgtgacaatggtcaagttcgacgataagaaatgcatgtacgacatctggaccttcgtgcccggctcccagccgggagagttcaccctgggcaagatcaagtccttccccggccacacttccagcctggtccgcgtggtctcgaccaactataatcagcatgctatggtgttcttcaagttcgtctttcagaatagagaggagttctacatcacactgtatggacgcaccaaggagctgacaagcgagctgaaagaaaacttcatcaggttttcaaagtccctggggctgcccgaaaatcatatcgtgttcccagtccccatcgaccagtgtattgatggt

SEQ ID NO: 23 - DNA, 642 bp, artificial; identical to SEQ ID NO: 21
  fusion polypeptide

SEQ ID NO: 24 - DNA, 1920 bp, artificial
  fusion polypeptide
gaagtccagctggtcgaatctggtggtggcctggtccagcctggtggatcactgagactgtcctgtgctgcttctggtttcaacatcaaggacacctacatccattgggtcagacaggcacctggcaagggactggaatgggtcgcccgaatctaccctacaaacggctacactcgctacgccgactccgtcaagggacgctttaccatctccgccgacacctctaaaaacaccgcctacctgcaaatgaatagtctgagggccgaggatactgctgtgtactactgctcacgatggggaggcgacggcttttacgctatggattactggggacagggaactctggtcactgtctcgagcgctagcaccaagggcccctccgtgttccccctggccccttgctcccggtccacctccgagtctaccgccgctctgggctgcctggtgaaagactacttccccgagcctgtgaccgtgagctggaactctggcgccctgacctccggcgtgcacaccttccctgccgtgctgcaatcctccggcctgtactccctgtcctccgtggtgacagtgccctcctccagcctgggcaccaagacctacacctgtaacgtggaccacaagccctccaacaccaaggtggacaagcgggtggaatctaaatacggccctccctgccccccctgccctgcccctgaagcggcgggcggaccttccgtgtttctgttccccccaaagcccaaggacaccctgatgatctcccggacccccgaagtgacctgcgtggtggtggacgtgtcccaggaagatccagaggtgcagttcaactggtatgttgacggcgtggaagtgcacaacgccaagaccaagcccagagaggaacagttcaactccacctaccgggtggtgtccgtgctgaccgtgctgcaccaggactggctgaacggcaaagagtacaagtgcaaggtgtccaacaagggcctgccctccagcatcgaaaagaccatctccaaggccaagggccagccccgcgagccccaggtgtacaccctgccccctagccaggaagagatgaccaagaaccaggtgtccctgacctgtctggtgaaaggcttctacccctccgacattgccgtggaatgggagtccaacggccagcccgagaacaactacaagaccaccccccctgtgctggactccgacggctccttcttcctgtactctcggctgacagtggataagtcccggtggcaggaaggcaatgtgttctcctgcagcgtgatgcacgaggccctgcacaaccactatacccagaagtccctgtccctgagcctgggcaagggcggtggaggatccgggggtgggggaagcggcggaggaggtagccaggactctactagtgatctgatcccggcaccgccactgtcaaaagtccctctgcaacaaaactttcaagacaatcagtttcacggcaaatggtatgtggtcggccaggccggaaacattaggctgcgggaggacaaggaccccatcaaaatgatggctaccatctacgagctgaaggaagacaaatcttatgatgtgacaatggtcaagttcgacgataagaaatgcatgtacgacatctggaccttcgtgcccggctcccagccgggagagttcaccctgggcaagatcaagtccttccccggccacacttccagcctggtccgcgtggtctcgaccaactataatcagcatgctatggtgttcttcaagttcgtctttcagaatagagaggagttctacatcacactgtatggacgcaccaaggagctgacaagcgagctgaaagaaaacttcatcaggttttcaaagtccctggggctgcccgaaaatcatatcgtgttcccagtccccatcgaccagtgtattgatggt

SEQ ID NO: 25 - DNA, 642 bp, artificial; identical to SEQ ID NO: 21
  fusion polypeptide

SEQ ID NO: 26 - DNA, 1341 bp, artificial
  fusion polypeptide
gaagtccagctggtcgaatctggtggtggcctggtccagcctggtggatcactgagactgtcctgtgctgcttctggtttcaacatcaaggacacctacatccattgggtcagacaggcacctggcaagggactggaatgggtcgcccgaatctaccctacaaacggctacactcgctacgccgactccgtcaagggacgctttaccatctccgccgacacctctaaaaacaccgcctacctgcaaatgaatagtctgagggccgaggatactgctgtgtactactgctcacgatggggaggcgacggcttttacgctatggattactggggacagggaactctggtcactgtctcgagcgctagcaccaagggcccctccgtgttccccctggccccttgctcccggtccacctccgagtctaccgccgctctgggctgcctggtgaaagactacttccccgagcctgtgaccgtgagctggaactctggcgccctgacctccggcgtgcacaccttccctgccgtgctgcaatcctccggcctgtactccctgtcctccgtggtgacagtgccctcctccagcctgggcaccaagacctacacctgtaacgtggaccacaagccctccaacaccaaggtggacaagcgggtggaatctaaatacggccctccctgccccccctgccctgcccctgaagcggcgggcggaccttccgtgtttctgttccccccaaagcccaaggacaccctgatgatctcccggacccccgaagtgacctgcgtggtggtggacgtgtcccaggaagatccagaggtgcagttcaactggtatgttgacggcgtggaagtgcacaacgccaagaccaagcccagagaggaacagttcaactccacctaccgggtggtgtccgtgctgaccgtgctgcaccaggactggctgaacggcaaagagtacaagtgcaaggtgtccaacaagggcctgccctccagcatcgaaaagaccatctccaaggccaagggccagccccgcgagccccaggtgtacaccctgccccctagccaggaagagatgaccaagaaccaggtgtccctgacctgtctggtgaaaggcttctacccctccgacattgccgtggaatgggagtccaacggccagcccgagaacaactacaagaccaccccccctgtgctggactccgacggctccttcttcctgtactctcggctgacagtggataagtcccggtggcaggaaggcaatgtgttctcctgcagcgtgatgcacgaggccctgcacaaccactatacccagaagtccctgtccctgagcctgggcaag

SEQ ID NO: 27 - DNA, 1062 bp, artificial
  fusion polypeptide
ctgtactctggggtgccttctcgattcagtggttctagatctggcaccgatttcacactgaccatttcttcactgcaacctgaggattttgccacctactactgtcagcagcactacacaacacctcccacatttggccagggcacaaaagtggagatcaaacggaccgtggcggcgccttctgtgttcattttccccccatctgatgaacagctgaaatctggcactgcttctgtggtctgtctgctgaacaacttctaccctagagaggccaaagtccagtggaaagtggacaatgctctgcagagtgggaattcccaggaatctgtcactgagcaggactctaaggatagcacatactccctgtcctctactctgacactgagcaaggctgattacgagaaacacaaagtgtacgcctgtgaagtcacacatcaggggctgtctagtcctgtgaccaaatccttcaataggggagagtgcggcggcggaggatccgggggtgggggaagcggcggaggaggtagccaggactctactagtgatctgatcccggcaccgccactgtcaaaagtccctctgcaacaaaactttcaagacaatcagtttcacggcaaatggtatgtggtcggccaggccggaaacattaggctgcgggaggacaaggaccccatcaaaatgatggctaccatctacgagctgaaggaagacaaatcttatgatgtgacaatggtcaagttcgacgataagaaatgcatgtacgacatctggaccttcgtgcccggctcccagccgggagagttcaccctgggcaagatcaagtccttccccggccacacttccagcctggtccgcgtggtctcgaccaactataatcagcatgctatggtgttcttcaagttcgtctttcagaatagagaggagttctacatcacactgtatggacgcaccaaggagctgacaagcgagctgaaagaaaacttcatcaggttttcaaagtccctggggctgcccgaaaatcatatcgtgttcccagtccccatcgaccagtgtattgatggt

SEQ ID NO: 28 - DNA, 1920 bp, artificial
  fusion polypeptide
caggactctactagtgatctgatcccggcaccgccactgtcaaaagtccctctgcaacaaaactttcaagacaatcagtttcacggcaaatggtatgtggtcggccaggccggaaacattaggctgcgggaggacaaggaccccatcaaaatgatggctaccatctacgagctgaaggaagacaaatcttatgatgtgacaatggtcaagttcgacgataagaaatgcatgtacgacatctggaccttcgtgcccggctcccagccgggagagttcaccctgggcaagatcaagtccttccccggccacacttccagcctggtccgcgtggtctcgaccaactataatcagcatgctatggtgttcttcaagttcgtctttcagaatagagaggagttctacatcacactgtatggacgcaccaaggagctgacaagcgagctgaaagaaaacttcatcaggttttcaaagtccctggggctgcccgaaaatcatatcgtgttcccagtccccatcgaccagtgtattgatggaggaggcggaggatccggcggaggaggaagtggcggaggaggaagtgaagtccagctggtcgaatctggtggtggcctggtccagcctggtggatcactgagactgtcctgtgctgcttctggtttcaacatcaaggacacctacatccattgggtcagacaggcacctggcaagggactggaatgggtcgcccgaatctaccctacaaacggctacactcgctacgccgactccgtcaagggacgctttaccatctccgccgacacctctaaaaacaccgcctacctgcagatgaatagtctgagggccgaggatactgctgtgtactactgctcacgatggggaggcgacggcttttacgctatggattactggggacagggaactctggtcactgtgtctagcgctagcaccaagggcccctccgtgttccccctggccccttgctcccggtccacctccgagtctaccgccgctctgggctgcctggtgaaagactacttccccgagcctgtgaccgtgagctggaactctggcgccctgacctccggcgtgcacaccttccctgccgtgctgcaatcctccggcctgtactccctgtcctccgtggtgacagtgccctcctccagcctgggcaccaagacctacacctgtaacgtggaccacaagccctccaacaccaaggtggacaagcgggtggaatctaaatacggccctccctgccccccctgccctgcccctgaagcggcgggcggaccttccgtgtttctgttccccccaaagcccaaggacaccctgatgatctcccggacccccgaagtgacctgcgtggtggtggacgtgtcccaggaagatccagaggtgcagttcaactggtatgttgacggcgtggaagtgcacaacgccaagaccaagcccagagaggaacagttcaactccacctaccgggtggtgtccgtgctgaccgtgctgcaccaggactggctgaacggcaaagagtacaagtgcaaggtgtccaacaagggcctgccctccagcatcgaaaagaccatctccaaggccaagggccagccccgcgagccccaggtgtacaccctgccccctagccaggaagagatgaccaagaaccaggtgtccctgacctgtctggtgaaaggcttctacccctccgacattgccgtggaatgggagtccaacggccagcccgagaacaactacaagaccaccccccctgtgctggactccgacggctccttcttcctgtactctcggctgacagtggataagtcccggtggcaggaaggcaatgtgttctcctgcagcgtgatgcacgaggccctgcacaaccactatacccagaagtccctgtccctgagcctgggcaag

SEQ ID NO: 29 - DNA, 642 bp, artificial; identical to SEQ ID NO: 21
  fusion polypeptide

SEQ ID NO: 30 - DNA, 1341 bp, artificial; identical to SEQ ID NO: 26
  fusion polypeptide

SEQ ID NO: 31 - DNA, 1221 bp, artificial
  fusion polypeptide
caggactctactagtgatctgatcccggcaccgccactgtcaaaagtccctctgcaacaaaactttcaagacaatcagtttcacggcaaatggtatgtggtcggccaggccggaaacattaggctgcgggaggacaaggaccccatcaaaatgatggctaccatctacgagctgaaggaagacaaatcttatgatgtgacaatggtcaagttcgacgataagaaatgcatgtacgacatctggaccttcgtgcccggctcccagccgggagagttcaccctgggcaagatcaagtccttccccggccacacttccagcctggtccgcgtggtctcgaccaactataatcagcatgctatggtgttcttcaagttcgtctttcagaatagagaggagttctacatcacactgtatggacgcaccaaggagctgacaagcgagctgaaagaaaacttcatcaggttttcaaagtccctggggctgcccgaaaatcatatcgtgttcccagtccccatcgaccagtgtattgatggaggaggcggaggatccggcggaggaggaagtggcggaggaggaagtgacatccagatgacacagtctccctcttccctgtccgcttctgtgggcgatcgagtgacaatcacctgtagggctagtcaggatgtgaatactgctgttgcttggtaccagcagaaaccaggaaaagcccctaaactgctgatctactctgcctcattcctgtactctggggtgccttctcgattcagtggttctagatctggcaccgatttcacactgaccatttcttcactgcaacctgaggattttgccacctactactgtcagcagcactacacaacacctcccacatttggccagggcacaaaagtggagatcaaacggaccgtggcggcgccttctgtgttcattttccccccatctgatgaacagctgaaatctggcactgcttctgtggtctgtctgctgaacaacttctaccctagagaggccaaagtccagtggaaagtggacaatgctctgcagagtgggaattcccaggaatctgtcactgagcaggactctaaggatagcacatactccctgtcctctactctgacactgagcaaggctgattacgagaaacacaaagtgtacgcctgtgaagtcacacatcaggggctgtctagtcctgtgaccaaatccttcaataggggagagtgc

SEQ ID NO: 32 - protein, 152 aa, artificial
  lipocalin mutein
ASDEEIQDVSGTWYLKAMTVDEGCRPWNIFSVTPMTLTTLEGGNLEAKVTMAIDGPAQEVKAVLEKTDEPGKYTADGGKHVAYIIRSHVKDHYIFYSEGVCDGSPVPGVWLVGRDPKNNLEALEDFEKAAGARGLSTESILIPRQSETSSPG

SEQ ID NO: 33 - protein, 152 aa, artificial
  lipocalin mutein
TSDEEIQDVSGTWYLKAMTVDEGCRPWNIFSVTPMTLTTLEGGNLEAKVTMAIDGPAQEVRAVLEKTDEPGKYTADGGKHDAYIIRSHVKDHYIFYSEGVCDGSPVPGVWLVGRDPENNLEALEDFEKTAGARGLSTESILIPRQSETSSPG

SEQ ID NO: 34 - protein, 152 aa, artificial
  lipocalin mutein
ASDEEIQDVSGTWYLKAMTVDEGCRPWNIFSVTPMTLTTLEGGNLEAKVTMAIDGPAQEVNAVLEKTDEPGKYTADGGKHVAYIIRSHVRDHYIFYSEGVCDGSPVPGVWLVGRDPENNLEALEDFEKTAGARGLSTESILIPRQSETSSPG

SEQ ID NO: 35 - protein, 152 aa, artificial
  lipocalin mutein
VSDEEIQDVSGTWYLKAMTVDEGCRPWNIFSVTPMTLTTLEGGNLEAKVTMAIDGPAQEVRAVLEKTDEPGKYTADGGKHVAYIIRSHVEDHYIFYSEGVCDGSPVPGVWLVGRDPENNLEALEDFEKTAGARGLSTESILIPRQSETSSPG

SEQ ID NO: 36 - protein, 152 aa, artificial
  lipocalin mutein
ASDEEIQDVSGTWYLKAMTVDEGCRPWNIFSVTPMTLSTLEGGNLEAKVTMAIDGPAQEVKAVLEKTDEPGKYTADGGKHVAYIIRSHVKDHYIFYSEGVCDGSPVPGVWLVGRDPKNNLEALEDFEKAAGARGLSTESILIPRQIETSSPG

SEQ ID NO: 37 - protein, 152 aa, artificial
  lipocalin mutein
ASDEEIQDVSGTWYLKAMTVDEGCRPWNIFSVTPMTLTTLEGGNLEAEVTMAIDGPAQEVKAVLEKADEPGKYTADGGKHVAYIIRSHVKDHYIFYSEGVCDGSPVPGVWLVGRDPKNNLEALEDFEKTAGARGLSTESILIPSQIETSSPG

SEQ ID NO: 38 - protein, 152 aa, artificial
  lipocalin mutein
TSDEEIQDVSGTWYLKAMTVDEGCRPWNIFSVTPMTLTTLEDGNLEAKVTMAIDGPAQEVKAVLEKADEPGKYTADGGKHVAYIIRSHVKDHYIFYSEGVCDGSPVPGVWLVGRDPKNNLEALEDFEKAAGARGLSTESILIPRQIETSSPG

SEQ ID NO: 39 - protein, 178 aa, artificial
  lipocalin mutein
QDSTSDLIPAPPLSKVPLQQNFQDNQFHGKWYVVGQAGNIKLREDKDPNKMMATIYELKEDKSYNVTGVTFDDKKCTYAISTFVPGSQPGEFTLGKIKSFPGHTSSLVRVVSTNYNQHAMVFFKFVFQNREEFYITLYGRTKELTSELKENFIRFSKSLGLPENHIVFPVPIDQCIDG

SEQ ID NO: 40 - protein, 178 aa, artificial
  lipocalin mutein
QDSTSDLIPAPPLSKVPLQQNFQDNQFHGKWYVVGQAGNIRLREDKDPNKMMATIYELKEDKSYDVTAVAFDDKKCTYDIWTFVPGSQPGEFTLGKIKSFPGHTSSLVRVVSTNYNQHAMVFFKFVFQNREEFYITLYGRTKELTSELKENFIRFSKSLGLPENHIVFPVPIDQCIDG

SEQ ID NO: 41 - protein, 178 aa, artificial
  lipocalin muein
QDSTSDLIPAPPLSKVPLQQNFQDNQFHGKWYVVGQAGNIKLREDKDPNKMMATIYELKEDKSYDVTAVAFDDKKCTYDIWTFVPGSQPGEFTLGKIKSFPGHTSSLVRVVSTNYNQHAMVFFKFVFQNREEFYITLYGRTKELTSELKENFIRFSKSLGLPENHIVFPVPIDQCIDG

SEQ ID NO: 42 - protein, 175 aa, artificial
  lipocalin mutein
QDSTSDLIPAPPLSKVPLQQNFQDNQFHGKWYVVGQAGNIKLREDSKMMATIYELKEDKSYDVTGVSFDDKKCTYAIMTFVPGSQPGEFTLGKIKSFPGHTSSLVRVVSTNYNQHAMVFFKFVFQNREEFYITLYGRTKELTSELKENFIRFSKSLGLPENHIVFPVPIDQCIDG

SEQ ID NO: 43 - protein, 178 aa, artificial
  lipocalin mutein
QDSTSDLIPAPPLSKVPLQQNFQDNQFHGKWYVVGQAGNIKLREDKDPVKMMATIYELKEDKSYDVTGVTFDDKKCRYDISTFVPGSQPGEFTFGKIKSFPGHTSSLVRVVSTNYNQHAMVFFKFVFQNREEFYITLYGRTKELTSELKENFIRFSKSLGLPENHIVFPVPIDQCIDG

SEQ ID NO: 44 - protein, 178 aa, artificial
  lipocalin mutein
QDSTSDLIPAPPLSKVPLQQNFQDNQFHGKWYVVGQAGNIRLREDKDPHKMMATIYELKEDKSYDVTGVTFDDKKCTYAISTFVPGSQPGEFTLGKIKSFPGHTSSLVRVVSTNYNQHAMVFFKFVFQNREEFYITLYGRTKELTSELKENFIRFSKSLGLPENHIVFPVPIDQCIDG

SEQ ID NO: 45 - protein, 178 aa, artificial
  lipocalin mutein
QDSTSDLIPAPPLSKVPLQQNFQDNQFHGKWYVVGQAGNIKLREDKDPNKMMATIYELKEDKSYDVTGVTFDDKKCTYAISTLVPGSQPGEFTFGKIKSFPGHTSSLVRVVSTNYNQHAMVFFKFVFQNREEFYITLYGRTKELTSELKENFIRFSKSLGLPENHIVFPVPIDQCIDG

SEQ ID NO: 46 - protein, 178 aa, artificial
  lipocalin mutein
QDSTSDLIPAPPLSKVPLQQNFQDNQFHGKWYVVGQAGNIRLREDKDPSKMMATIYELKEDKSYDVTAVTFDDKKCNYAISTFVPGSQPGEFTLGKIKSFPGHTSSLVRVVSTNYNQHAMVFFKFVFQNREEFYITLYGRTKELTSELKENFIRFSKSLGLPENHIVFPVPIDQCIDG

SEQ ID NO: 47 - protein, 448 aa, artificial
  reference antibody
QVQLQQWGAGLLKPSETLSLTCAVYGGSFSGYYWSWIRQSPEKGLEWIGEINHGGYVTYNPSLESRVTISVDTSKNQFSLKLSSVTAADTAVYYCARDYGPGNYDWYFDLWGRGTLVTVSSASTKGPSVFPLAPCSRSTSESTAALGCLVKDYFPEPVTVSWNSGALTSGVHTFPAVLQSSGLYSLSSVVTVPSSSLGTKTYTCNVDHKPSNTKVDKRVESKYGPPCPPCPAPEFLGGPSVFLFPPKPKDTLMISRTPEVTCVVVDVSQEDPEVQFNWYVDGVEVHNAKTKPREEQFNSTYRVVSVLTVLHQDWLNGKEYKCKVSNKGLPSSIEKTISKAKGQPREPQVYTLPPSQEEMTKNQVSLTCLVKGFYPSDIAVEWESNGQPENNYKTTPPVLDSDGSFFLYSRLTVDKSRWQEGNVFSCSVMHEALHNHYTQKSLSLSLGK

SEQ ID NO: 48 - protein, 216 aa, artificial
  reference antibody
EIVLTQSPATLSLSPGERATLSCRASQSVSSYLAWYQQKPGQAPRLLIYDASNRATGIPARFSGSGSGTDFTLTISSLEPEDFAVYYCQQRSNWPPALTFGGGTKVEIKRTVAAPSVFIFPPSDEQLKSGTASVVCLLNNFYPREAKVQWKVDNALQSGNSQESVTEQDSKDSTYSLSSTLTLSKADYEKHKVYACEVTHQGLSSPVTKSFNRGEC

SEQ ID NO: 49 - protein, 442 aa, artificial
  reference antibody
EVQLVQSGAEVKKPGESLRISCKGSGYSFSTYWISWVRQMPGKGLEWMGKIYPGDSYTNYSPSFQGQVTISADKSISTAYLQWSSLKASDTAMYYCARGYGIFDYWGQGTLVTVSSASTKGPSVFPLAPCSRSTSESTAALGCLVKDYFPEPVTVSWNSGALTSGVHTFPAVLQSSGLYSLSSVVTVPSSNFGTQTYTCNVDHKPSNTKVDKTVERKCCVECPPCPAPPVAGPSVFLFPPKPKDTLMISRTPEVTCVVVDVSHEDPEVQFNWYVDGVEVHNAKTKPREEQFNSTFRVVSVLTVVHQDWLNGKEYKCKVSNKGLPAPIEKTISKTKGQPREPQVYTLPPSREEMTKNQVSLTCLVKGFYPSDIAVEWESNGQPENNYKTTPPMLDSDGSFFLYSKLTVDKSRWQQGNVFSCSVMHEALHNHYTQKSLSLSPGK

SEQ ID NO: 50 - protein, 214 aa, artificial
  reference antibody
SYELTQPPSVSVSPGQTASITCSGDNIGDQYAHWYQQKPGQSPVLVIYQDKNRPSGIPERFSGSNSGNTATLTISGTQAMDEADYYCATYTGFGSLAVFGGGTKLTVLGQPKAAPSVTLFPPSSEELQANKATLVCLISDFYPGAVTVAWKADSSPVKAGVETTTPSKQSNNKYAASSYLSLTPEQWKSHRSYSCQVTHEGSTVEKTVAPTECS

SEQ ID NO: 51 - protein, 447 aa, artificial; identical to SEQ ID NO: 11
  Trastuzumab-IgG4 S228P FALA (Heavy chain)

SEQ ID NO: 52 - protein, 214 aa, artificial; identical to SEQ ID NO: 4
  Trastuzumab-IgG4 S228P FALA (Light chain)